European Patent Application EP 4 268 846 A1, published November 1, 2023. Title: IMMUNOGENIC FORMULATION CONTAINING ONE OR MORE MODIFIED BCG STRAINS EXPRESSING A SARS-COV-2 PROTEIN, USEFUL FOR PREVENTING, TREATING OR ATTENUATING THE DEVELOPMENT OF COVID-19. Applicant: Pontificia Universidad Católica de Chile Fundación Copec-UC. The sequence listing filed with the application follows.

SEQUENCE LISTING (4 sequences)

SEQ ID NO: 1 - DNA, 1272 bp, SARS-CoV-2
ttcgaaatgtctgataatggaccccaaaatcagcgaaatgcaccccgcattacgtttggtggaccctcagattcaactggcagtaaccagaatggagaacgcagtggggcgcgatcaaaacaacgtcggccccaaggtttacccaataatactgcgtcttggttcaccgctctcactcaacatggcaaggaagaccttaaattccctcgaggacaaggcgttccaattaacaccaatagcagtccagatgaccaaattggctactaccgaagagctaccagacgaattcgtggtggtgacggtaaaatgaaagatctcagtccaagatggtatttctactacctaggaactgggccagaagctggacttccctatggtgctaacaaagacggcatcatatgggttgcaactgagggagccttgaatacaccaaaagatcacattggcacccgcaatcctgctaacaatgctgcaatcgtgctacaacttcctcaaggaacaacattgccaaaaggcttctacgcagaagggagcagaggcggcagtcaagcctcttctcgttcctcatcacgtagtcgcaacagttcaagaaattcaactccaggcagcagtaggggaacttctcctgctagaatggctggcaatggcggtgatgctgctcttgctttgctgctgcttgacagattgaaccagcttgagagcaaaatgtctggtaaaggccaacaacaacaaggccaaactgtcactaagaaatctgctgctgaggcttctaagaagcctcggcaaaaacgtactgccactaaagcatacaatgtaacacaagctttcggcagacgtggtccagaacaaacccaaggaaattttggggaccaggaactaatcagacaaggaactgattacaaacattggccgcaaattgcacaatttgcccccagcgcttcagcgttcttcggaatgtcgcgcattggcatggaagtcacaccttcgggaacgtggttgacctacacaggtgccatcaaattggatgacaaagatccaaatttcaaagatcaagtcattttgctgaataagcatattgacgcatacaaaacattcccaccaacagagcctaaaaaggacaaaaagaagaaggctgatgaaactcaagccttaccgcagagacagaagaaacagcaaactgtgactcttcttcctgctgcagatttggatgatttctccaaacaattgcaacaatccatgagcagtgctgactcaactcaggcctaaatcgat

SEQ ID NO: 2 - DNA, 240 bp, SARS-CoV-2
ttcgaaatgtactcattcgtttcggaagagacaggtacgttaatagttaatagcgtacttctttttcttgctttcgtggtattcttgctagttacactagccatccttactgcgcttcgattgtgtgcgtactgctgcaatattgttaacgtgagtcttgtaaaaccttctttttacgtttactctcgtgttaaaaatctgaattcttctagagttcctgatcttctggtctaaatcgat

SEQ ID NO: 3 - DNA, 681 bp, SARS-CoV-2
ttcgaaatggcagattccaacggtactattaccgttgaagagcttaaaaagctccttgaacaatggaacctagtaataggtttcctattccttacatggatttgtcttctacaatttgcctatgccaacaggaataggtttttgtatataattaagttaattttcctctggctgttatggccagtaactttagcttgttttgtgcttgctgctgtttacagaataaattggatcaccggtggaattgctatcgcaatggcttgtcttgtaggcttgatgtggctcagctacttcattgcttctttcagactgtttgcgcgtacgcgttccatgtggtcattcaatccagaaactaacattcttctcaacgtgccactccatggcactattctgaccagaccgcttctagaaagtgaactcgtaatcggagctgtgatccttcgtggacatcttcgtattgctggacaccatctaggacgctgtgacatcaaggacctgcctaaagaaatcactgttgctacatcacgaacgctttcttattacaaattgggagcttcgcagcgtgtagcaggtgactcaggttttgctgcatacagtcgctacaggattggcaactataaattaaacacagaccattccagtagcagtgacaatattgctttgcttgtacagtaaatcgat

SEQ ID NO: 4 - DNA, 3651 bp, SARS-CoV-2
caattgatgtttgtttttcttgttttattgccactagtctctagtcagtgtgttaatcttacaaccagaactcaattaccccctgcatacactaattctttcacacgtggtgtttattaccctgacaaagttttcagatcctcagttttacattcaactcaggacttgttcttacctttcttttccaatgttacttggttccatgctatacatgtctctgggaccaatggtactaagaggtttgataaccctgtcctaccatttaatgatggtgtttattttgcttccactgagaagtctaacataataagaggctggatttttggtactactttagattcgaagacccagtccctacttattgttaataacgctactaatgttgttattaaagtctgtgaatttcaattttgtaatgatccatttttgggtgtttattaccacaaaaacaacaaaagttggatggaaagtgagttcagagtttattctagtgcgaataattgcacttttgaatatgtctctcagccttttcttatggaccttgaaggaaaacagggtaatttcaaaaatcttagggaatttgtgtttaagaatattgatggttattttaaaatatattctaagcacacgcctattaatttagtgcgtgatctccctcagggtttttcggctttagaaccattggtagatttgccaataggtattaacatcactaggtttcaaactttacttgctttacatagaagttatttgactcctggtgattcttcttcaggttggacagctggtgctgcagcttattatgtgggttatcttcaacctaggacttttctattaaaatataatgaaaatggaaccattacagatgctgtagactgtgcacttgaccctctctcagaaacaaagtgtacgttgaaatccttcactgtagaaaaaggaatctatcaaacttctaactttagagtccaaccaacagaatctattgttagatttcctaatattacaaacttgtgcccttttggtgaagtttttaacgccaccagatttgcatctgtttatgcttggaacaggaagagaatcagcaactgtgttgctgattattctgtcctatataattccgcatcattttccacttttaagtgttatggagtgtctcctactaaattaaatgatctctgctttactaatgtctatgcagattcatttgtaattagaggtgatgaagtcagacaaatcgctccagggcaaactggaaagattgctgattataattataaattaccagatgattttacaggctgcgttatagcttggaattctaacaatcttgattctaaggttggtggtaattataattacctgtatagattgtttaggaagtctaatctcaaaccttttgagagagatatttcaactgaaatctatcaggccggtagcacaccttgtaatggtgttgaaggttttaattgttactttcctttacaatcatatggtttccaacccactaatggtgttggttaccaaccatacagagtagtagtactttcttttgaacttctacatgcaccagcaactgtttgtggacctaaaaagtctactaatttggttaaaaacaaatgtgtcaatttcaacttcaatggtttaacaggcacaggtgttcttactgagtctaacaaaaagtttctgcctttccaacaatttggcagagacattgctgacactactgatgctgtccgtgatccacagacacttgagattcttgacattacaccatgttcttttggtggtgtcagtgttataacaccaggaacaaatacttctaaccaggttgctgttctttatcaggatgttaactgcacagaagtccctgttgctattcatgcagatcaacttactcctacttggcgtgtttattctacaggttctaatgtttttcaaacacgtgcaggctgtttaataggggctgaacatgtcaacaactcatatgagtgtgacatacccattggtgcaggtatatgcgctagttatcagactcagactaattctcctcggcgggcacgtagtgtagctagtcaatccatcattgcctacactatgtcacttggtgcagaaaattcagttgcttactctaataactctattgccatacccacaaattttactattagtgttaccacagaaattctaccagtgtctatgaccaagacatcagtagattgtacaatgtacatttgtggtgattcaactgaatgcagcaatcttttgttgcaatatggcagtttttgtacacaattaaaccgtgctttaactggaatagctgttgaacaagacaaaaacacccaagaagtttttgcacaagtcaaacaaatttacaaaacaccaccaattaaagattttggtggttttaatttttcacaaatattaccagatccatcaaaaccaagcaagaggtcatttattgaagatctacttttcaacaaagtgacacttgcagatgctggcttcatcaaacaatatggtgattgccttggtgatattgctgctagagacctcatttgtgcacaaaagtttaacggccttactgttttgccacctttgctcacagatgaaatgattgctcaatacacttctgcactgttagcgggtacaatcacttctggttggacctttggtgcaggtgctgcattacaaataccatttgctatgcaaatggcttataggtttaatggtattggagttacacagaatgttctctatgagaaccaaaaattgattgccaaccaatttaatagtgctattggcaaaattcaagactcactttcttccacagcaagtgcacttggaaaacttcaagatgtggtcaaccaaaatgcacaagctttaaacacgcttgttaaacaacttagctccaattttggtgcaatttcaagtgttttaaatgatatcctttcacgtcttgacaaagttgaggctgaagtgcaaattgataggttgatcacaggcagacttcaaagtttgcagacatatgtgactcaacaattaattagagctgcagaaatcagagcttctgctaatcttgctgctactaaaatgtcagagtgtgtacttggacaatcaaaaagagttgatttttgtggaaagggctatcatcttatgtccttccctcagtcagcacctcatggtgtagtcttcttgcatgtgacttatgtccctgcacaagaaaagaacttcacaactgctcctgccatttgtcatgatggaaaagcacactttcctcgtgaaggtgtctttgtttcaaatggcacacactggtttgtaacacaaaggaatttttatgaaccacaaatcattactacagacaacacatttgtgtctggtaactgtgatgttgtaataggaattgtcaacaacacagtttatgatcctttgcaacctgaattagactcattcaaggaggagttagataaatattttaagaatcatacatcaccagatgttgatttaggtgacatctctggcattaatgcttcagttgtaaacattcaaaaagaaattgaccgcctcaatgaggttgccaagaatttaaatgaatctctcatcgatctccaagaacttggaaagtatgagcagtatataaaatggccacttaag